European Patent Specification EP 2 692 853 B1, published May 6, 2026. Title: Membrane-based sorting incubator, membrane-based sorting kit and method for isolating stem cells using thereof. Applicant: National Institute for Longevity Sciences. The sequence listing filed with the application follows.

SEQUENCE LISTING (76 sequences)

SEQ ID NO: 1 - DNA, 20 bp, Artificial Sequence
  Canine forward primer for Sox2
agctagtctccaagcgacga

SEQ ID NO: 2 - DNA, 20 bp, Artificial Sequence
  Canine reverse primer for Sox2
ccacgtttgcaactgtccta

SEQ ID NO: 3 - DNA, 20 bp, Artificial Sequence
  Canine forward primer for Bmi1
cactcccgttcagtctcctc

SEQ ID NO: 4 - DNA, 20 bp, Artificial Sequence
  Canine reverse primer for Bmi1
ccagatgaagttgctgacga

SEQ ID NO: 5 - DNA, 20 bp, Artificial Sequence
  Canine forward primer for CXCR4
ctgtggcaaactggtacttc

SEQ ID NO: 6 - DNA, 20 bp, Artificial Sequence
  Canine reverse primer for CXCR4
tcaacaggagggcaggtatc

SEQ ID NO: 7 - DNA, 20 bp, Artificial Sequence
  Canine forward primer for Stat3
gtggtgacggagaagcaaca

SEQ ID NO: 8 - DNA, 20 bp, Artificial Sequence
  Canine reverse primer for Stat3
ttctgtctggtcaccgactg

SEQ ID NO: 9 - DNA, 20 bp, Artificial Sequence
  Canine forward primer for GM-CSF
gcagaacctgcttttcttgg

SEQ ID NO: 10 - DNA, 20 bp, Artificial Sequence
  Canine reverse primer for GM-CSF
ccctcagggtcaaacacttc

SEQ ID NO: 11 - DNA, 20 bp, Artificial Sequence
  Canine forward primer for MMP3
ccctctgattcctccaatga

SEQ ID NO: 12 - DNA, 20 bp, Artificial Sequence
  Canine reverse primer for MMP3
ggatggccaaaatgaagaga

SEQ ID NO: 13 - DNA, 20 bp, Artificial Sequence
  Canine forward primer for VEGF-A
ctacctccaccatgccaagt

SEQ ID NO: 14 - DNA, 20 bp, Artificial Sequence
  Canine reverse primer for VEGF-A
acgcaggatggcttgaagat

SEQ ID NO: 15 - DNA, 20 bp, Artificial Sequence
  Canine forward primer for BDNF
gttggccgacacttttgaac

SEQ ID NO: 16 - DNA, 20 bp, Artificial Sequence
  Canine reverse primer for BDNF
cctcatcgacatgtttgcag

SEQ ID NO: 17 - DNA, 19 bp, Artificial Sequence
  Canine forward primer for GDNF
gccgagcagtgactcaaac

SEQ ID NO: 18 - DNA, 19 bp, Artificial Sequence
  Canine reverse primer for GDNF
tctcgggtgaccttttcag

SEQ ID NO: 19 - DNA, 20 bp, Artificial Sequence
  Canine forward primer for NGF
caacaggactcacaggagca

SEQ ID NO: 20 - DNA, 20 bp, Artificial Sequence
  Canine reverse primer for NGF
atgttcacctctcccagcac

SEQ ID NO: 21 - DNA, 20 bp, Artificial Sequence
  Canine forward primer for beta-actin
aagtaccccattgagcacgg

SEQ ID NO: 22 - DNA, 20 bp, Artificial Sequence
  Canine reverse primer for beta-actin
atcacgatgccagtggtgcg

SEQ ID NO: 23 - DNA, 19 bp, Artificial Sequence
  Human forward primer for Oct4
cagtgcccgaaacccacac

SEQ ID NO: 24 - DNA, 20 bp, Artificial Sequence
  Human reverse primer for Oct4
ggagacccagcagcctcaaa

SEQ ID NO: 25 - DNA, 20 bp, Artificial Sequence
  Human forward primer for Nanog
cagaaggcctcagcacctac

SEQ ID NO: 26 - DNA, 20 bp, Artificial Sequence
  Human reverse primer for Nanog
attgttccaggtctggttgc

SEQ ID NO: 27 - DNA, 20 bp, Artificial Sequence
  Human forward primer for Sox2
aatgccttcatggtgtggtc

SEQ ID NO: 28 - DNA, 20 bp, Artificial Sequence
  Human reverse primer for Sox2
cggggccggtatttataatc

SEQ ID NO: 29 - DNA, 20 bp, Artificial Sequence
  Human forward primer for Rex1
tggacacgtctgtgctcttc

SEQ ID NO: 30 - DNA, 20 bp, Artificial Sequence
  Human reverse primer for Rex2
ctcgaaccttccagatcacc

SEQ ID NO: 31 - DNA, 20 bp, Artificial Sequence
  Human forward primer for Stat3
gtggtgacggagaagcagca

SEQ ID NO: 32 - DNA, 20 bp, Artificial Sequence
  Human reverse primer for Stat3
ttctgcctggtcactgactg

SEQ ID NO: 33 - DNA, 20 bp, Artificial Sequence
  Human forward primer for CXCR4
ccgtggcaaactggtacttt

SEQ ID NO: 34 - DNA, 20 bp, Artificial Sequence
  Human reverse primer for CXCR4
tcagcaggagggcagggatc

SEQ ID NO: 35 - DNA, 20 bp, Artificial Sequence
  Human forward primer for GM-CSF
gcctggagctgtacaagcag

SEQ ID NO: 36 - DNA, 20 bp, Artificial Sequence
  Human reverse primer for GM-CSF
cagcagtcaaaggggatgac

SEQ ID NO: 37 - DNA, 20 bp, Artificial Sequence
  Human forward primer for MMP3
cctcaggaagcttgaacctg

SEQ ID NO: 38 - DNA, 20 bp, Artificial Sequence
  Human reverse primer for MMP3
gggaaacctagggtgtggat

SEQ ID NO: 39 - DNA, 20 bp, Artificial Sequence
  Human forward primer for VEGF-A
atggcagaaggagaccagaa

SEQ ID NO: 40 - DNA, 20 bp, Artificial Sequence
  Human reverse primer for VEGF-A
atggcgatgttgaactcctc

SEQ ID NO: 41 - DNA, 20 bp, Artificial Sequence
  Human forward primer for BDNF
aaacatccgaggacaaggtg

SEQ ID NO: 42 - DNA, 20 bp, Artificial Sequence
  Human reverse primer for BDNF
cgtgtacaagtctgcgtcct

SEQ ID NO: 43 - DNA, 20 bp, Artificial Sequence
  Human forward primer for GDNF
ccaacccagagaattccaga

SEQ ID NO: 44 - DNA, 20 bp, Artificial Sequence
  Human reverse primer for GDNF
agccgctgcagtacctaaaa

SEQ ID NO: 45 - DNA, 20 bp, Artificial Sequence
  Human forward primer for NGF
atacaggcggaaccacactc

SEQ ID NO: 46 - DNA, 19 bp, Artificial Sequence
  Human reverse primer for NGF
gcctggggtccacagtaat

SEQ ID NO: 47 - DNA, 20 bp, Artificial Sequence
  Human forward primer for NT-3
agactcgctcaattccctca

SEQ ID NO: 48 - DNA, 20 bp, Artificial Sequence
  Human reverse primer for NT-3
ggtgtccattgcaatcactg

SEQ ID NO: 49 - DNA, 20 bp, Artificial Sequence
  Human forward primer for beta-actin
ggacttcgagcaagagatgg

SEQ ID NO: 50 - DNA, 20 bp, Artificial Sequence
  Human reverse primer for beta-actin
agcactgtgttggcgtacag

SEQ ID NO: 51 - DNA, 19 bp, Artificial Sequence
  Porcine forward primer for Nanog
ccccgaagcatccatttcc

SEQ ID NO: 52 - DNA, 22 bp, Artificial Sequence
  Porcine reverse primer for Nanog
cgagggtctcagcagatgacat

SEQ ID NO: 53 - DNA, 20 bp, Artificial Sequence
  Porcine forward primer for Sox2
aatgccttcatggtgtggtc

SEQ ID NO: 54 - DNA, 20 bp, Artificial Sequence
  Porcine reverse primer for Sox2
cggggccggtatttataatc

SEQ ID NO: 55 - DNA, 20 bp, Artificial Sequence
  Porcine forward primer for Stat3
gtggtgacagagaagcagca

SEQ ID NO: 56 - DNA, 20 bp, Artificial Sequence
  Porcine reverse primer for Stat3
ttctgcctggtcactgactg

SEQ ID NO: 57 - DNA, 18 bp, Artificial Sequence
  Porcine forward primer for Tert
caggtgtaccgcctcctg

SEQ ID NO: 58 - DNA, 20 bp, Artificial Sequence
  Porcine reverse primer for Tert
ccagatgcagtcttgcactt

SEQ ID NO: 59 - DNA, 20 bp, Artificial Sequence
  Porcine forward primer for Bmi1
atatttacggtgcccagcag

SEQ ID NO: 60 - DNA, 20 bp, Artificial Sequence
  Porcine reverse primer for Bmi1
gaagtggcccattccttctc

SEQ ID NO: 61 - DNA, 20 bp, Artificial Sequence
  Porcine forward primer for CXCR4
ccgtggcaaactggtacttt

SEQ ID NO: 62 - DNA, 20 bp, Artificial Sequence
  Porcine reverse primer for CXCR4
tcaacaggagggcaggtatc

SEQ ID NO: 63 - DNA, 20 bp, Artificial Sequence
  Porcine forward primer for GM-CSF
gccctgagccttctaaacaa

SEQ ID NO: 64 - DNA, 20 bp, Artificial Sequence
  Porcine reverse primer for GM-CSF
gtgctgctcatagtgcttgg

SEQ ID NO: 65 - DNA, 20 bp, Artificial Sequence
  Porcine forward primer for MMP3
acccagatgtggagttcctg

SEQ ID NO: 66 - DNA, 21 bp, Artificial Sequence
  Porcine reverse primer for MMP3
ggagtcacttcctcccagatt

SEQ ID NO: 67 - DNA, 20 bp, Artificial Sequence
  Porcine forward primer for VEGF-A
atggcagaaggagaccagaa

SEQ ID NO: 68 - DNA, 20 bp, Artificial Sequence
  Porcine reverse primer for VEGF-A
atggcgatgttgaactcctc

SEQ ID NO: 69 - DNA, 20 bp, Artificial Sequence
  Porcine forward primer for BDNF
ttcaagaggcctgacatcgt

SEQ ID NO: 70 - DNA, 20 bp, Artificial Sequence
  Porcine reverse primer for BDNF
agaagaggaggctccaaagg

SEQ ID NO: 71 - DNA, 20 bp, Artificial Sequence
  Porcine forward primer for GDNF
acggccatacacctcaatgt

SEQ ID NO: 72 - DNA, 20 bp, Artificial Sequence
  Porcine reverse primer for GDNF
ccgtctgtttttggacaggt

SEQ ID NO: 73 - DNA, 20 bp, Artificial Sequence
  Porcine forward primer for NGF
tggtgttgggagaggtgaat

SEQ ID NO: 74 - DNA, 19 bp, Artificial Sequence
  Porcine reverse primer for NGF
ccgtgtcgattcggataaa

SEQ ID NO: 75 - DNA, 20 bp, Artificial Sequence
  Porcine forward primer for beta-actin
ctcttccagccctccttcct

SEQ ID NO: 76 - DNA, 20 bp, Artificial Sequence
  Porcine reverse primer for beta-actin
acgtcgcacttcatgatcga